European Patent Application EP 4 324 472 A2, published February 21, 2024. Title: Novel peptides and combination of peptides for use in immunotherapy against prostate cancer and other cancers. Applicant: immatics biotechnologies GmbH. The sequence listing filed with the application follows.

SEQUENCE LISTING (61 sequences)

SEQ ID NO: 1 - protein, 10 aa, Homo sapiens
VTAQIGIVAV

SEQ ID NO: 2 - protein, 9 aa, Homo sapiens
SMLGEEIQL

SEQ ID NO: 3 - protein, 9 aa, Homo sapiens
HLLEDIAHV

SEQ ID NO: 4 - protein, 9 aa, Homo sapiens
ALLTFVWKL

SEQ ID NO: 5 - protein, 9 aa, Homo sapiens
KIFSRLIYI

SEQ ID NO: 6 - protein, 9 aa, Homo sapiens
ALLESRVNL

SEQ ID NO: 7 - protein, 11 aa, Homo sapiens
TLLQVVGVVSV

SEQ ID NO: 8 - protein, 9 aa, Homo sapiens
LLDFSLADA

SEQ ID NO: 9 - protein, 13 aa, Homo sapiens
GMLNEAEGKAIKL

SEQ ID NO: 10 - protein, 9 aa, Homo sapiens
TLWRGPVVV

SEQ ID NO: 11 - protein, 9 aa, Homo sapiens
YLEEECPAT

SEQ ID NO: 12 - protein, 9 aa, Homo sapiens
SLNEEIAFL

SEQ ID NO: 13 - protein, 9 aa, Homo sapiens
AMAPNHAVV

SEQ ID NO: 14 - protein, 10 aa, Homo sapiens
KMDEASAQLL

SEQ ID NO: 15 - protein, 11 aa, Homo sapiens
KMDEASAQLLA

SEQ ID NO: 16 - protein, 9 aa, Homo sapiens
KMDEASAQL

SEQ ID NO: 17 - protein, 9 aa, Homo sapiens
RLGIKPESV

SEQ ID NO: 18 - protein, 9 aa, Homo sapiens
GLSEFTEYL

SEQ ID NO: 19 - protein, 9 aa, Homo sapiens
LLPPPPLLA

SEQ ID NO: 20 - protein, 9 aa, Homo sapiens
SLLSHQVLL

SEQ ID NO: 21 - protein, 9 aa, Homo sapiens
YLNDSLRHV

SEQ ID NO: 22 - protein, 9 aa, Homo sapiens
SLYDSIAFI

SEQ ID NO: 23 - protein, 11 aa, Homo sapiens
AVAGADVIITV

SEQ ID NO: 24 - protein, 9 aa, Homo sapiens
SYNDALLTF

SEQ ID NO: 25 - protein, 9 aa, Homo sapiens
IYEPYLAMF

SEQ ID NO: 26 - protein, 11 aa, Homo sapiens
RYADDTFTPAF

SEQ ID NO: 27 - protein, 9 aa, Homo sapiens
GYLQGLVSF

SEQ ID NO: 28 - protein, 9 aa, Homo sapiens
YYAKEIHKF

SEQ ID NO: 29 - protein, 9 aa, Homo sapiens
RYGSPINTF

SEQ ID NO: 30 - protein, 9 aa, Homo sapiens
SYSPAHARL

SEQ ID NO: 31 - protein, 9 aa, Homo sapiens
AYTSPPSFF

SEQ ID NO: 32 - protein, 11 aa, Homo sapiens
PYQLNASLFTF

SEQ ID NO: 33 - protein, 9 aa, Homo sapiens
QYGKDFLTL

SEQ ID NO: 34 - protein, 11 aa, Homo sapiens
AFSPDSHYLLF

SEQ ID NO: 35 - protein, 9 aa, Homo sapiens
IYTRVTYYL

SEQ ID NO: 36 - protein, 9 aa, Homo sapiens
RYMWINQEL

SEQ ID NO: 37 - protein, 9 aa, Homo sapiens
RYLQDLLAW

SEQ ID NO: 38 - protein, 9 aa, Homo sapiens
VYSDKLWIF

SEQ ID NO: 39 - protein, 9 aa, Homo sapiens
SYIDVAVKL

SEQ ID NO: 40 - protein, 9 aa, Homo sapiens
RTFSPTYGL

SEQ ID NO: 41 - protein, 9 aa, Homo sapiens
RYLQKIEEF

SEQ ID NO: 42 - protein, 9 aa, Homo sapiens
TYIGQGYII

SEQ ID NO: 43 - protein, 9 aa, Homo sapiens
AYIKNGQLF

SEQ ID NO: 44 - protein, 11 aa, Homo sapiens
VYNTVSEGTHF

SEQ ID NO: 45 - protein, 9 aa, Homo sapiens
RYFKTPRKF

SEQ ID NO: 46 - protein, 9 aa, Homo sapiens
VYEEILHQI

SEQ ID NO: 47 - protein, 9 aa, Homo sapiens
SYTPVLNQF

SEQ ID NO: 48 - protein, 10 aa, Homo sapiens
AWAPKPYHKF

SEQ ID NO: 49 - protein, 11 aa, Homo sapiens
SLFHPEDTGQV

SEQ ID NO: 50 - protein, 9 aa, Homo sapiens
TLGPASFLV

SEQ ID NO: 51 - protein, 9 aa, Homo sapiens
AMFDKKVQL

SEQ ID NO: 52 - protein, 9 aa, Homo sapiens
ALGDLVQSV

SEQ ID NO: 53 - protein, 11 aa, Homo sapiens
YLLKDKGEYTL

SEQ ID NO: 54 - protein, 9 aa, Homo sapiens
AYSEKVTEF

SEQ ID NO: 55 - protein, 9 aa, Homo sapiens
LYFEKGEYF

SEQ ID NO: 56 - protein, 11 aa, Homo sapiens
LFHPEDTGQVF

SEQ ID NO: 57 - protein, 9 aa, Homo sapiens
KYADKIYSI

SEQ ID NO: 58 - protein, 9 aa, Homo sapiens
GYIDKVRQL

SEQ ID NO: 59 - protein, 9 aa, Homo sapiens
IYPDVTYAF

SEQ ID NO: 60 - protein, 10 aa, Homo sapiens
ELAGIGILTV

SEQ ID NO: 61 - protein, 9 aa, Homo sapiens
YLLPAIVHI